European Patent Application EP 4 806 903 A1, published September 16, 2026. Title: 一种全过程靶向多肽、其药物复合物、递药系统及其应用. Applicant: 复旦大学. The sequence listing filed with the application follows.

SEQUENCE LISTING (4 sequences)

SEQ ID NO: 1 - protein, 7 aa, synthetic construct
SNTRVAP

SEQ ID NO: 2 - protein, 7 aa, synthetic construct
PAVRTNS

SEQ ID NO: 3 - protein, 7 aa, synthetic construct
  VARIANT 1..7: note = D type amino acid
PAVRTNS

SEQ ID NO: 4 - protein, 7 aa, synthetic construct
  VARIANT 1..7: note = D type amino acid
SNTRVAP